European Patent Specification EP 4 015 631 B1, published February 18, 2026. Title: Novel processes for the production of oligonucleotides. Applicant: GlaxoSmithKline Intellectual Property Development Limited. The sequence listing filed with the application follows.

SEQUENCE LISTING (101 sequences)

SEQ ID NO: 1 - DNA, 20 bp, Artificial Sequence
  Example 1 desired product oligonucleotide sequence ("target")
ggccaaacctcggcttacct

SEQ ID NO: 2 - DNA, 23 bp, Artificial Sequence
  Example 1-4, 6, 10 and 11 template oligonucleotide sequence
tttaggtaagccgaggtttggcc

SEQ ID NO: 3 - protein, 487 aa, enterobacteria phage T4
MILKILNEIASIGSTKQKQAILEKNKDNELLKRVYRLTYSRGLQYYIKKWPKPGIATQSFGMLTLTDMLDFIEFTLATRKLTGNAAIEELTGYITDGKKDDVEVLRRVMMRDLECGASVSIANKVWPGLIPEQPQMLASSYDEKGINKNIKFPAFAQLKADGARCFAEVRGDELDDVRLLSRAGNEYLGLDLLKEELIKMTAEARQIHPEGVLIDGELVYHEQVKKEPEGLDFLFDAYPENSKAKEFAEVAESRTASNGIANKSLKGTISEKEAQCMKFQVWDYVPLVEIYSLPAFRLKYDVRFSKLEQMTSGYDKVILIENQVVNNLDEAKVIYKKYIDQGLEGIILKNIDGLWENARSKNLYKFKEVIDVDLKIVGIYPHRKDPTKAGGFILESECGKIKVNAGSGLKDKAGVKSHELDRTRIMENQNYYIGKILECECNGWLKSDGRTDYVKLFLPIAIRLREDKTKANTFEDVFGDFHEVTGL

SEQ ID NO: 4 - protein, 488 aa, Artificial Sequence
  Wild type T4 DNA ligase protein sequence (when fused to CBD)
GSILKILNEIASIGSTKQKQAILEKNKDNELLKRVYRLTYSRGLQYYIKKWPKPGIATQSFGMLTLTDMLDFIEFTLATRKLTGNAAIEELTGYITDGKKDDVEVLRRVMMRDLECGASVSIANKVWPGLIPEQPQMLASSYDEKGINKNIKFPAFAQLKADGARCFAEVRGDELDDVRLLSRAGNEYLGLDLLKEELIKMTAEARQIHPEGVLIDGELVYHEQVKKEPEGLDFLFDAYPENSKAKEFAEVAESRTASNGIANKSLKGTISEKEAQCMKFQVWDYVPLVEIYSLPAFRLKYDVRFSKLEQMTSGYDKVILIENQVVNNLDEAKVIYKKYIDQGLEGIILKNIDGLWENARSKNLYKFKEVIDVDLKIVGIYPHRKDPTKAGGFILESECGKIKVNAGSGLKDKAGVKSHELDRTRIMENQNYYIGKILECECNGWLKSDGRTDYVKLFLPIAIRLREDKTKANTFEDVFGDFHEVTGL

SEQ ID NO: 5 - RNA, 20 nt, Artificial Sequence
  Example 2 target sequence
ggccaaaccucggcuuaccu

SEQ ID NO: 6 - protein, 482 aa, Enterobacteria phase CC31
MILDIINEIASIGSTKEKEAIIRRHKDNELLKRVFRMTYDGKLQYYIKKWDTRPKGDIHLTLEDMLYLLEEKLAKRVVTGNAAKEKLEIALSQTSDADAEVVKKVLLRDLRCGASRSIANKVWKNLIPEQPQMLASSYDEKGIEKNIKFPAFAQLKADGARAFAEVRGDELDDVKILSRAGNEYLGLDLLKQQLIEMTKEARERHPGGVMIDGELVYHASTLPAGPLDDIFGDLPELSKAKEFKEESRTMSNGLANKSLKGTISAKEAAGMKFQVWDYVPLDVVYSEGKQSGFAYDVRFRALELMVQGYSQMILIENHIVHNLDEAKVIYRKYVDEGLEGIILKNIGAFWENTRSKNLYKFKEVITIDLRIVDIYEHSKQPGKAGGFYLESECGLIKVKAGSGLKDKPGKDAHELDRTRIWENKNDYIGGVLESECNGWLAAEGRTDYVKLFLPIAIKMRRDKDVANTFADIWGDFHEVTGL

SEQ ID NO: 7 - protein, 483 aa, Artificial Sequence
  Wild-type Enterobacteria phage CC31 DNA ligase protein sequence (when fused to CBD)
GSILDIINEIASIGSTKEKEAIIRRHKDNELLKRVFRMTYDGKLQYYIKKWDTRPKGDIHLTLEDMLYLLEEKLAKRVVTGNAAKEKLEIALSQTSDADAEVVKKVLLRDLRCGASRSIANKVWKNLIPEQPQMLASSYDEKGIEKNIKFPAFAQLKADGARAFAEVRGDELDDVKILSRAGNEYLGLDLLKQQLIEMTKEARERHPGGVMIDGELVYHASTLPAGPLDDIFGDLPELSKAKEFKEESRTMSNGLANKSLKGTISAKEAAGMKFQVWDYVPLDVVYSEGKQSGFAYDVRFRALELMVQGYSQMILIENHIVHNLDEAKVIYRKYVDEGLEGIILKNIGAFWENTRSKNLYKFKEVITIDLRIVDIYEHSKQPGKAGGFYLESECGLIKVKAGSGLKDKPGKDAHELDRTRIWENKNDYIGGVLESECNGWLAAEGRTDYVKLFLPIAIKMRRDKDVANTFADIWGDFHEVTGL

SEQ ID NO: 8 - protein, 497 aa, Shigella phage Shf125875
MILDILNQIAAIGSTKTKQEILKKNKDNKLLERVYRLTYARGIQYYIKKWPGPGERSQAYGLLELDDMLDFIEFTLATRKLTGNAAIKELMGYIADGKPDDVEVLRRVMMRDLEVGASVSIANKVWPGLIQLQPQMLASAYDEKLITKNIKWPAFAQLKADGARCFAEVRDDGVQFFSRAGNEYHGLTLLADELMEMTKEARERHPNGVLIDGELVYHSFDIKKAVSSGNDLSFLFGDNEESEEVQVADRSTSNGLANKSLQGTISPKEAEGMVLQAWDYVPLDEVYSDGKIKGQKYDVRFAALENMAEGFKRIEPIENQLVHNLDEAKVVYKKYVDQGLEGIILKNRDSYWENKRSKNLIKFKEVIDIALEVVGYYEHSKDPNKLGGVELVSRCRRITTDCGSGFKDTTHKTVDGVKVLIPLDERHDLDRERLMAEAREGKLIGRIADCECNGWVHSKGREGTVGIFLPIIKGFRFDKTEADSFEDVFGPWSQTGL

SEQ ID NO: 9 - protein, 498 aa, Artificial Sequence
  Wild-type Shigella phage Shf125875 DNA ligase protein sequence (when fused to CBD)
GSILDILNQIAAIGSTKTKQEILKKNKDNKLLERVYRLTYARGIQYYIKKWPGPGERSQAYGLLELDDMLDFIEFTLATRKLTGNAAIKELMGYIADGKPDDVEVLRRVMMRDLEVGASVSIANKVWPGLIQLQPQMLASAYDEKLITKNIKWPAFAQLKADGARCFAEVRDDGVQFFSRAGNEYHGLTLLADELMEMTKEARERHPNGVLIDGELVYHSFDIKKAVSSGNDLSFLFGDNEESEEVQVADRSTSNGLANKSLQGTISPKEAEGMVLQAWDYVPLDEVYSDGKIKGQKYDVRFAALENMAEGFKRIEPIENQLVHNLDEAKVVYKKYVDQGLEGIILKNRDSYWENKRSKNLIKFKEVIDIALEVVGYYEHSKDPNKLGGVELVSRCRRITTDCGSGFKDTTHKTVDGVKVLIPLDERHDLDRERLMAEAREGKLIGRIADCECNGWVHSKGREGTVGIFLPIIKGFRFDKTEADSFEDVFGPWSQTGL

SEQ ID NO: 10 - protein, 487 aa, Artificial Sequence
  Mutant ligase (T4 backbone) protein sequence
MILKILNEIASIGSTKQKQAILEKNKDNELLKRVYRLTYSRGLQYYIKKWPKPGIATQSFGMLTLTDMLDFIEFTLATRKLTGNAAIEELTGYITDGKKDDVEVLRRVMMRDLECGASVSIANKVWPGLIPEQPQMLASSYDEKGINKNIKFPAFAQLKADGARCFAEVRGDELDDVRLLSRAGNEYLGLDLLKEELIKMTAEARQIHPEGVLIDGELVYHEQVKKEPEGLDFLFDAYPENSKAKEFAEVAESRTASNGIANKSLKGTISEKEAQCMKFQVWDYVPLVEIYSLPAFRLKYDVRFSKLEQMTSGYDKVILIENQVVNNLDEAKVIYKKYIDQGLEGIILKNIDGLWENARSKNLYKFKRVIDVDLKIVGIYPHRKDPTKAGGFILESECGKIKVNAGSGLKDKAGVKSHELDRTRIMENQNYYIGKILECECNGWLKSDGRTDYVKLFLPIAIRLREDKTKANTFEDVFGDFHEVTGL

SEQ ID NO: 11 - protein, 487 aa, Artificial Sequence
  Mutant ligase (T4 backbone) protein sequence
MILKILNEIASIGSTKQKQAILEKNKDNELLKRVYRLTYSRGLQYYIKKWPKPGIATQSFGMLTLTDMLDFIEFTLATRKLTGNAAIEELTGYITDGKKDDVEVLRRVMMRDLECGASVSIANKVWPGLIPEQPQMLASSYDEKGINKNIKFPAFAQLKADGARCFAEVRGDELDDVRLLSRAGNEYLGLDLLKEELIKMTAEARQIHPEGVLIDGELVYHEQVKKEPEGLDFLFDAYPENSKAKEFAEVAESRTASNGIANKSLKGTISEKEAQCMKFQVWDYVPLVEIYSLPAFRLKYDVRFSKLEQMTSGYDKVILIENQVVNNLDEAKVIYKKYIDQGLEGIILKNIDGLWENARSKNLYKFKGVIDVDLKIVGIYPHRKDPTKAGGFILESECGKIKVNAGSGLKDKAGVKSHELDRTRIMENQNYYIGKILECECNGWLKSDGRTDYVKLFLPIAIRLREDKTKANTFEDVFGDFHEVTGL

SEQ ID NO: 12 - protein, 487 aa, Artificial Sequence
  Mutant ligase (T4 backbone) protein sequence
MILKILNEIASIGSTKQKQAILEKNKDNELLKRVYRLTYSRGLQYYIKKWPKPGIATQSFGMLTLTDMLDFIEFTLATRKLTGNAAIEELTGYITDGKKDDVEVLRRVMMRDLECGASVSIANKVWPGLIPEQPQMLASSYDEKGINKNIKFPAFAQLKADGARCFAEVRGDELDDVRLLSRAGNEYLGLDLLKEELIKMTAEARQIHPEGVLIDGELVYHEQVKKEPEGLDFLFDAYPENSKAKEFAEVAESRTASNGIANKSLKGTISEKEAQCMKFQVWDYVPLVEIYSLPAFRLKYDVRFSKLEQMTSGYDKVILIENQVVNNLDEAKVIYKKYIDQGLEGIILKNIDGLWENARSKNLYKFKKVIDVDLKIVGIYPHRKDPTKAGGFILESECGKIKVNAGSGLKDKAGVKSHELDRTRIMENQNYYIGKILECECNGWLKSDGRTDYVKLFLPIAIRLREDKTKANTFEDVFGDFHEVTGL

SEQ ID NO: 13 - protein, 487 aa, Artificial Sequence
  Mutant ligase (T4 backbone) protein sequence
MILKILNEIASIGSTKQKQAILEKNKDNELLKRVYRLTYSRGLQYYIKKWPKPGIATQSFGMLTLTDMLDFIEFTLATRKLTGNAAIEELTGYITDGKKDDVEVLRRVMMRDLECGASVSIANKVWPGLIPEQPQMLASSYDEKGINKNIKFPAFAQLKADGARCFAEVRGDELDDVRLLSRAGNEYLGLDLLKEELIKMTAEARQIHPEGVLIDGELVYHEQVKKEPEGLDFLFDAYPENSKAKEFAEVAESRTASNGIANKSLKGTISEKEAQCMKFQVWDYVPLVEIYSLPAFRLKYDVRFSKLEQMTSGYDKVILIENQVVNNLDEAKVIYKKYIDQGLEGIILKNIDGLWENARSKNLYKFKEVILVDLKIVGIYPHRKDPTKAGGFILESECGKIKVNAGSGLKDKAGVKSHELDRTRIMENQNYYIGKILECECNGWLKSDGRTDYVKLFLPIAIRLREDKTKANTFEDVFGDFHEVTGL

SEQ ID NO: 14 - protein, 487 aa, Artificial Sequence
  Mutant ligase (T4 backbone) protein sequence
MILKILNEIASIGSTKQKQAILEKNKDNELLKRVYRLTYSRGLQYYIKKWPKPGIATQSFGMLTLTDMLDFIEFTLATRKLTGNAAIEELTGYITDGKKDDVEVLRRVMMRDLECGASVSIANKVWPGLIPEQPQMLASSYDEKGINKNIKFPAFAQLKADGARCFAEVRGDELDDVRLLSRAGNEYLGLDLLKEELIKMTAEARQIHPEGVLIDGELVYHEQVKKEPEGLDFLFDAYPENSKAKEFAEVAESRTASNGIANKSLKGTISEKEAQCMKFQVWDYVPLVEIYSLPAFRLKYDVRFSKLEQMTSGYDKVILIENQVVNNLDEAKVIYKKYIDQGLEGIILKNIDGLWENARSKNLYKFKEVIKVDLKIVGIYPHRKDPTKAGGFILESECGKIKVNAGSGLKDKAGVKSHELDRTRIMENQNYYIGKILECECNGWLKSDGRTDYVKLFLPIAIRLREDKTKANTFEDVFGDFHEVTGL

SEQ ID NO: 15 - protein, 487 aa, Artificial Sequence
  Mutant ligase (T4 backbone) protein sequence
MILKILNEIASIGSTKQKQAILEKNKDNELLKRVYRLTYSRGLQYYIKKWPKPGIATQSFGMLTLTDMLDFIEFTLATRKLTGNAAIEELTGYITDGKKDDVEVLRRVMMRDLECGASVSIANKVWPGLIPEQPQMLASSYDEKGINKNIKFPAFAQLKADGARCFAEVRGDELDDVRLLSRAGNEYLGLDLLKEELIKMTAEARQIHPEGVLIDGELVYHEQVKKEPEGLDFLFDAYPENSKAKEFAEVAESRTASNGIANKSLKGTISEKEAQCMKFQVWDYVPLVEIYSLPAFRLKYDVRFSKLEQMTSGYDKVILIENQVVNNLDEAKVIYKKYIDQGLEGIILKNIDGLWENARSKNLYKFKEVIQVDLKIVGIYPHRKDPTKAGGFILESECGKIKVNAGSGLKDKAGVKSHELDRTRIMENQNYYIGKILECECNGWLKSDGRTDYVKLFLPIAIRLREDKTKANTFEDVFGDFHEVTGL

SEQ ID NO: 16 - protein, 487 aa, Artificial Sequence
  Mutant ligase (T4 backbone) protein sequence
MILKILNEIASIGSTKQKQAILEKNKDNELLKRVYRLTYSRGLQYYIKKWPKPGIATQSFGMLTLTDMLDFIEFTLATRKLTGNAAIEELTGYITDGKKDDVEVLRRVMMRDLECGASVSIANKVWPGLIPEQPQMLASSYDEKGINKNIKFPAFAQLKADGARCFAEVRGDELDDVRLLSRAGNEYLGLDLLKEELIKMTAEARQIHPEGVLIDGELVYHEQVKKEPEGLDFLFDAYPENSKAKEFAEVAESRTASNGIANKSLKGTISEKEAQCMKFQVWDYVPLVEIYSLPAFRLKYDVRFSKLEQMTSGYDKVILIENQVVNNLDEAKVIYKKYIDQGLEGIILKNIDGLWENARSKNLYKFKEVIVVDLKIVGIYPHRKDPTKAGGFILESECGKIKVNAGSGLKDKAGVKSHELDRTRIMENQNYYIGKILECECNGWLKSDGRTDYVKLFLPIAIRLREDKTKANTFEDVFGDFHEVTGL

SEQ ID NO: 17 - protein, 487 aa, Artificial Sequence
  Mutant ligase (T4 backbone) protein sequence
MILKILNEIASIGSTKQKQAILEKNKDNELLKRVYRLTYSRGLQYYIKKWPKPGIATQSFGMLTLTDMLDFIEFTLATRKLTGNAAIEELTGYITDGKKDDVEVLRRVMMRDLECGASVSIANKVWPGLIPEQPQMLASSYDEKGINKNIKFPAFAQLKADGARCFAEVRGDELDDVRLLSRAGNEYLGLDLLKEELIKMTAEARQIHPEGVLIDGELVYHEQVKKEPEGLDFLFDAYPENSKAKEFAEVAESRTASNGIANKSLKGTISEKEAQCMKFQVWDYVPLVEIYSLPAFRLKYDVRFSKLEQMTSGYDKVILIENQVVNNLDEAKVIYKKYIDQGLEGIILKNIDGLWENARSKNLYKFKEVIRVDLKIVGIYPHRKDPTKAGGFILESECGKIKVNAGSGLKDKAGVKSHELDRTRIMENQNYYIGKILECECNGWLKSDGRTDYVKLFLPIAIRLREDKTKANTFEDVFGDFHEVTGL

SEQ ID NO: 18 - protein, 487 aa, Artificial Sequence
  Mutant ligase (T4 backbone) protein sequence
MILKILNEIASIGSTKQKQAILEKNKDNELLKRVYRLTYSRGLQYYIKKWPKPGIATQSFGMLTLTDMLDFIEFTLATRKLTGNAAIEELTGYITDGKKDDVEVLRRVMMRDLECGASVSIANKVWPGLIPEQPQMLASSYDEKGINKNIKFPAFAQLKADGARCFAEVRGDELDDVRLLSRAGNEYLGLDLLKEELIKMTAEARQIHPEGVLIDGELVYHEQVKKEPEGLDFLFDAYPENSKAKEFAEVAESRTASNGIANKSLKGTISEKEAQCMKFQVWDYVPLVEIYSLPAFRLKYDVRFSKLEQMTSGYDKVILIENQVVNNLDEAKVIYKKYIDQGLEGIILKNIDGLWENARSKNLYKFKEAIDVDLKIVGIYPHRKDPTKAGGFILESECGKIKVNAGSGLKDKAGVKSHELDRTRIMENQNYYIGKILECECNGWLKSDGRTDYVKLFLPIAIRLREDKTKANTFEDVFGDFHEVTGL

SEQ ID NO: 19 - protein, 487 aa, Artificial Sequence
  Mutant ligase (T4 backbone) protein sequence
MILKILNEIASIGSTKQKQAILEKNKDNELLKRVYRLTYSRGLQYYIKKWPKPGIATQSFGMLTLTDMLDFIEFTLATRKLTGNAAIEELTGYITDGKKDDVEVLRRVMMRDLECGASVSIANKVWPGLIPEQPQMLASSYDEKGINKNIKFPAFAQLKADGARCFAEVRGDELDDVRLLSRAGNEYLGLDLLKEELIKMTAEARQIHPEGVLIDGELVYHEQVKKEPEGLDFLFDAYPENSKAKEFAEVAESRTASNGIANKSLKGTISEKEAQCMKFQVWDYVPLVEIYSLPAFRLKYDVRFSKLEQMTSGYDKVILIENQVVNNLDEAKVIYKKYIDQGLEGIILKNIDGLWENARSKNLYKFKEKIDVDLKIVGIYPHRKDPTKAGGFILESECGKIKVNAGSGLKDKAGVKSHELDRTRIMENQNYYIGKILECECNGWLKSDGRTDYVKLFLPIAIRLREDKTKANTFEDVFGDFHEVTGL

SEQ ID NO: 20 - protein, 487 aa, Artificial Sequence
  Mutant ligase (T4 backbone) protein sequence
MILKILNEIASIGSTKQKQAILEKNKDNELLKRVYRLTYSRGLQYYIKKWPKPGIATQSFGMLTLTDMLDFIEFTLATRKLTGNAAIEELTGYITDGKKDDVEVLRRVMMRDLECGASVSIANKVWPGLIPEQPQMLASSYDEKGINKNIKFPAFAQLKADGARCFAEVRGDELDDVRLLSRAGNEYLGLDLLKEELIKMTAEARQIHPEGVLIDGELVYHEQVKKEPEGLDFLFDAYPENSKAKEFAEVAESRTASNGIANKSLKGTISEKEAQCMKFQVWDYVPLVEIYSLPAFRLKYDVRFSKLEQMTSGYDKVILIENQVVNNLDEAKVIYKKYIDQGLEGIILKNIDGLWENARSKNLYKFKRVIVVDLKIVGIYPHRKDPTKAGGFILESECGKIKVNAGSGLKDKAGVKSHELDRTRIMENQNYYIGKILECECNGWLKSDGRTDYVKLFLPIAIRLREDKTKANTFEDVFGDFHEVTGL

SEQ ID NO: 21 - protein, 487 aa, Artificial Sequence
  Mutant ligase (T4 backbone) protein sequence
MILKILNEIASIGSTKQKQAILEKNKDNELLKRVYRLTYSRGLQYYIKKWPKPGIATQSFGMLTLTDMLDFIEFTLATRKLTGNAAIEELTGYITDGKKDDVEVLRRVMMRDLECGASVSIANKVWPGLIPEQPQMLASSYDEKGINKNIKFPAFAQLKADGARCFAEVRGDELDDVRLLSRAGNEYLGLDLLKEELIKMTAEARQIHPEGVLIDGELVYHEQVKKEPEGLDFLFDAYPENSKAKEFAEVAESRTASNGIANKSLKGTISEKEAQCMKFQVWDYVPLVEIYSLPAFRLKYDVRFSKLEQMTSGYDKVILIENQVVNNLDEAKVIYKKYIDQGLEGIILKNIDGLWENARSKNLYKFKKVIEVDLKIVGIYPHRKDPTKAGGFILESECGKIKVNAGSGLKDKAGVKSHELDRTRIMENQNYYIGKILECECNGWLKSDGRTDYVKLFLPIAIRLREDKTKANTFEDVFGDFHEVTGL

SEQ ID NO: 22 - protein, 487 aa, Artificial Sequence
  Mutant ligase (T4 backbone) protein sequence
MILKILNEIASIGSTKQKQAILEKNKDNELLKRVYRLTYSRGLQYYIKKWPKPGIATQSFGMLTLTDMLDFIEFTLATRKLTGNAAIEELTGYITDGKKDDVEVLRRVMMRDLECGASVSIANKVWPGLIPEQPQMLASSYDEKGINKNIKFPAFAQLKADGARCFAEVRGDELDDVRLLSRAGNEYLGLDLLKEELIKMTAEARQIHPEGVLIDGELVYHEQVKKEPEGLDFLFDAYPENSKAKEFAEVAESRTASNGIANKSLKGTISEKEAQCMKFQVWDYVPLVEIYSLPAFRLKYDVRFSKLEQMTSGYDKVILIENQVVNNLDEAKVIYKKYIDQGLEGIILKNIDGLWENARSKNLYKFKKVIHVDLKIVGIYPHRKDPTKAGGFILESECGKIKVNAGSGLKDKAGVKSHELDRTRIMENQNYYIGKILECECNGWLKSDGRTDYVKLFLPIAIRLREDKTKANTFEDVFGDFHEVTGL

SEQ ID NO: 23 - protein, 482 aa, Artificial Sequence
  Mutant ligase (Enterobacteria phage CC31 backbone - clone A4) protein sequence
MILDIINEIASIGSTKEKEAIIRRHKDNELLKRVFRMTYDGKLQYYIKKWDTRPKGDIHLTLEDMLYLLEEKLAKRVVTGNAAKEKLEIALSQTSDADAEVVKKVLLRDLRCGASRSIANKVWKNLIPEQPQMLASSYDEKGIEKNIKFPAFAQLKADGARAFAEVRGDELDDVKILSRAGNEYLGLDLLKQQLIEMTKEARERHPGGVMIDGELVYHASTLPAGPLDDIFGDLPELSKAKEFKEESRTMSNGLANKSLKGTISAKEAAGMKFQVWDYVPLDVVYSEGKQSGFAYDVRFRALELMVQGYSQMILIENHIVHNLDEAKVIYRKYVDEGLEGIILKNIGAFWENTRSKNLYKFKRVIVIDLRIVDIYEHSKQPGKAGGFYLESECGLIKVKAGSGLKDKPGKDAHELDRTRIWENKNDYIGGVLESECNGWLAAEGRTDYVKLFLPIAIKMRRDKDVANTFADIWGDFHEVTGL

SEQ ID NO: 24 - protein, 482 aa, Artificial Sequence
  Mutant ligase (Enterobacteria phage CC31 backbone) protein sequence
MILDIINEIASIGSTKEKEAIIRRHKDNELLKRVFRMTYDGKLQYYIKKWDTRPKGDIHLTLEDMLYLLEEKLAKRVVTGNAAKEKLEIALSQTSDADAEVVKKVLLRDLRCGASRSIANKVWKNLIPEQPQMLASSYDEKGIEKNIKFPAFAQLKADGARAFAEVRGDELDDVKILSRAGNEYLGLDLLKQQLIEMTKEARERHPGGVMIDGELVYHASTLPAGPLDDIFGDLPELSKAKEFKEESRTMSNGLANKSLKGTISAKEAAGMKFQVWDYVPLDVVYSEGKQSGFAYDVRFRALELMVQGYSQMILIENHIVHNLDEAKVIYRKYVDEGLEGIILKNIGAFWENTRSKNLYKFKKVIKIDLRIVDIYEHSKQPGKAGGFYLESECGLIKVKAGSGLKDKPGKDAHELDRTRIWENKNDYIGGVLESECNGWLAAEGRTDYVKLFLPIAIKMRRDKDVANTFADIWGDFHEVTGL

SEQ ID NO: 25 - protein, 482 aa, Artificial Sequence
  Mutant ligase (Enterobacteria phage CC31 backbone) protein sequence
MILDIINEIASIGSTKEKEAIIRRHKDNELLKRVFRMTYDGKLQYYIKKWDTRPKGDIHLTLEDMLYLLEEKLAKRVVTGNAAKEKLEIALSQTSDADAEVVKKVLLRDLRCGASRSIANKVWKNLIPEQPQMLASSYDEKGIEKNIKFPAFAQLKADGARAFAEVRGDELDDVKILSRAGNEYLGLDLLKQQLIEMTKEARERHPGGVMIDGELVYHASTLPAGPLDDIFGDLPELSKAKEFKEESRTMSNGLANKSLKGTISAKEAAGMKFQVWDYVPLDVVYSEGKQSGFAYDVRFRALELMVQGYSQMILIENHIVHNLDEAKVIYRKYVDEGLEGIILKNIGAFWENTRSKNLYKFKGVIFIDLRIVDIYEHSKQPGKAGGFYLESECGLIKVKAGSGLKDKPGKDAHELDRTRIWENKNDYIGGVLESECNGWLAAEGRTDYVKLFLPIAIKMRRDKDVANTFADIWGDFHEVTGL

SEQ ID NO: 26 - protein, 482 aa, Artificial Sequence
  Mutant ligase (Enterobacteria phage CC31 backbone) protein sequence
MILDIINEIASIGSTKEKEAIIRRHKDNELLKRVFRMTYDGKLQYYIKKWDTRPKGDIHLTLEDMLYLLEEKLAKRVVTGNAAKEKLEIALSQTSDADAEVVKKVLLRDLRCGASRSIANKVWKNLIPEQPQMLASSYDEKGIEKNIKFPAFAQLKADGARAFAEVRGDELDDVKILSRAGNEYLGLDLLKQQLIEMTKEARERHPGGVMIDGELVYHASTLPAGPLDDIFGDLPELSKAKEFKEESRTMSNGLANKSLKGTISAKEAAGMKFQVWDYVPLDVVYSEGKQSGFAYDVRFRALELMVQGYSQMILIENHIVHNLDEAKVIYRKYVDEGLEGIILKNIGAFWENTRSKNLYKFKGVILIDLRIVDIYEHSKQPGKAGGFYLESECGLIKVKAGSGLKDKPGKDAHELDRTRIWENKNDYIGGVLESECNGWLAAEGRTDYVKLFLPIAIKMRRDKDVANTFADIWGDFHEVTGL

SEQ ID NO: 27 - protein, 482 aa, Artificial Sequence
  Mutant ligase (Enterobacteria phage CC31 backbone) protein sequence
MILDIINEIASIGSTKEKEAIIRRHKDNELLKRVFRMTYDGKLQYYIKKWDTRPKGDIHLTLEDMLYLLEEKLAKRVVTGNAAKEKLEIALSQTSDADAEVVKKVLLRDLRCGASRSIANKVWKNLIPEQPQMLASSYDEKGIEKNIKFPAFAQLKADGARAFAEVRGDELDDVKILSRAGNEYLGLDLLKQQLIEMTKEARERHPGGVMIDGELVYHASTLPAGPLDDIFGDLPELSKAKEFKEESRTMSNGLANKSLKGTISAKEAAGMKFQVWDYVPLDVVYSEGKQSGFAYDVRFRALELMVQGYSQMILIENHIVHNLDEAKVIYRKYVDEGLEGIILKNIGAFWENTRSKNLYKFKRVIFIDLRIVDIYEHSKQPGKAGGFYLESECGLIKVKAGSGLKDKPGKDAHELDRTRIWENKNDYIGGVLESECNGWLAAEGRTDYVKLFLPIAIKMRRDKDVANTFADIWGDFHEVTGL

SEQ ID NO: 28 - protein, 497 aa, Artificial Sequence
  Mutant ligase (Shigella phage Shf125875 backbone) protein sequence
MILDILNQIAAIGSTKTKQEILKKNKDNKLLERVYRLTYARGIQYYIKKWPGPGERSQAYGLLELDDMLDFIEFTLATRKLTGNAAIKELMGYIADGKPDDVEVLRRVMMRDLEVGASVSIANKVWPGLIQLQPQMLASAYDEKLITKNIKWPAFAQLKADGARCFAEVRDDGVQFFSRAGNEYHGLTLLADELMEMTKEARERHPNGVLIDGELVYHSFDIKKAVSSGNDLSFLFGDNEESEEVQVADRSTSNGLANKSLQGTISPKEAEGMVLQAWDYVPLDEVYSDGKIKGQKYDVRFAALENMAEGFKRIEPIENQLVHNLDEAKVVYKKYVDQGLEGIILKNRDSYWENKRSKNLIKFKRVIVIALEVVGYYEHSKDPNKLGGVELVSRCRRITTDCGSGFKDTTHKTVDGVKVLIPLDERHDLDRERLMAEAREGKLIGRIADCECNGWVHSKGREGTVGIFLPIIKGFRFDKTEADSFEDVFGPWSQTGL

SEQ ID NO: 29 - protein, 298 aa, Paramecium bursaria Chlorella virus PBCV-1
MAITKPLLAATLENIEDVQFPCLATPKIDGIRSVKQTQMLSRTFKPIRNSVMNRLLTELLPEGSDGEISIEGATFQDTTSAVMTGHKMYNAKFSYYWFDYVTDDPLKKYIDRVEDMKNYITVHPHILEHAQVKIIPLIPVEINNITELLQYERDVLSKGFEGVMIRKPDGKYKFGRSTLKEGILLKMKQFKDAEATIISMTALFKNTNTKTKDNFGYSKRSTHKSGKVEEDVMGSIEVDYDGVVFSIGTGFDADQRRDFWQNKESYIGKMVKFKYFEMGSKDCPRFPVFIGIRHEEDR

SEQ ID NO: 30 - DNA, 23 bp, Artificial Sequence
  Example 5, 8 and 9 template oligonucleotide sequence
tttggtgcgaagcagactgaggc

SEQ ID NO: 31 - DNA, 23 bp, Artificial Sequence
  Example 5 template oligonucleotide sequence
tttggtgcgaagcagagtgaggc

SEQ ID NO: 32 - DNA, 23 bp, Artificial Sequence
  Example 5 template oligonucleotide sequence
tttggtgcgaagcagattgaggc

SEQ ID NO: 33 - DNA, 23 bp, Artificial Sequence
  Example 5 template oligonucleotide sequence
tttggtgcgaagcagaatgaggc

SEQ ID NO: 34 - DNA, 23 bp, Artificial Sequence
  Example 5 template oligonucleotide sequence
tttggtgcgaagcagtctgaggc

SEQ ID NO: 35 - DNA, 23 bp, Artificial Sequence
  Example 5 template oligonucleotide sequence
tttggtgcgaagcagtgtgaggc

SEQ ID NO: 36 - DNA, 23 bp, Artificial Sequence
  Example 5 template oligonucleotide sequence
tttggtgcgaagcagtttgaggc

SEQ ID NO: 37 - DNA, 23 bp, Artificial Sequence
  Example 5 template oligonucleotide sequence
tttggtgcgaagcagtatgaggc

SEQ ID NO: 38 - DNA, 23 bp, Artificial Sequence
  Example 5 template oligonucleotide sequence
tttggtgcgaagcagcctgaggc

SEQ ID NO: 39 - DNA, 23 bp, Artificial Sequence
  Example 5 template oligonucleotide sequence
tttggtgcgaagcagcgtgaggc

SEQ ID NO: 40 - DNA, 23 bp, Artificial Sequence
  Example 5 template oligonucleotide sequence
tttggtgcgaagcagcttgaggc

SEQ ID NO: 41 - DNA, 23 bp, Artificial Sequence
  Example 5 template oligonucleotide sequence
tttggtgcgaagcagcatgaggc

SEQ ID NO: 42 - DNA, 23 bp, Artificial Sequence
  Example 5 template oligonucleotide sequence
tttggtgcgaagcaggctgaggc

SEQ ID NO: 43 - DNA, 23 bp, Artificial Sequence
  Example 5 template oligonucleotide sequence
tttggtgcgaagcagggtgaggc

SEQ ID NO: 44 - DNA, 23 bp, Artificial Sequence
  Example 5 template oligonucleotide sequence
tttggtgcgaagcaggttgaggc

SEQ ID NO: 45 - DNA, 23 bp, Artificial Sequence
  Example 5 template oligonucleotide sequence
tttggtgcgaagcaggatgaggc

SEQ ID NO: 46 - DNA, 20 bp, Artificial Sequence
  Example 14 "20 mer" oligonucleotide sequence
gccucagtctgcttcgcacc

SEQ ID NO: 47 - DNA, 36 bp, Artificial Sequence
  Example 7 template oligonucleotide sequence
tttggtgcgaagcagaaggtaagccgaggtttggcc

SEQ ID NO: 48 - protein, 298 aa, Paramecium bursaria Chlorella virus NE-JV-4
MAITKPLLAATLENIEDVQFPCLATPKIDGIRSVKQTQMLSRTFKPIRNSVMNRLLTELLPEGSDGEISIEGATFQDTTSAVMTGHKMYNAKFSYYWFDYVTDDPLKKYSDRVEDMKNYITAHPHILDHEQVKIIPLIPVEINNITELLQYERDVLSKGFEGVMIRKPDGKYKFGRSTLKEGILLKMKQFKDAEATIISMTALFKNTNTKTKDNFGYSKRSTHKNGKVEEDVMGSIEVDYDGVVFSIGTGFDADQRRDFWQNKESYIGKMVKFKYFEMGSKDCPRFPVFIGIRHEEDH

SEQ ID NO: 49 - protein, 298 aa, Paramecium bursaria Chlorella virus NYs1
MTIAKPLLAATLENLDDVKFPCLVTPKIDGIRSLKQQHMLSRTFKPIRNSVMNKLLSELLPEGADGEICIEDSTFQATTSAVMTGHKVYDEKFSYYWFDYVVDDPLKSYTDRVNDMKKYVDDHPHILEHEQVKIIPLIPVEINNIDELSQYERDVLAKGFEGVMIRRPDGKYKFGRSTLKEGILLKMKQFKDAEATIISMSPRLKNTNAKSKDNLGYSKRSTHKSGKVEEETMGSIEVDYDGVVFSIGTGFDDEQRKHFWENKDSYIGKLLKFKYFEMGSKDAPRFPVFIGIRHEEDC

SEQ ID NO: 50 - protein, 301 aa, Paramecium bursaria Chlorella virus NE-JV-1
MTAIQKPLLAASFKKLTVADVKYPVFATPKLDGIRALKIDGAFVSRTFKPIRNRAIADALQDLLPNGSDGEILSGSTFQDASSAVMTAKAGIGANTIFYWFDYVKDDPNKPYLDRMTDMENYLKERPEILNDDRIKIVPLIPKKIETKDELDTFEKICLDQGFEGVMIRSGAGKYKFGRSTEKEGILIKIKQFEDDEAVVIGFTPMQTNTNDKSMNELGDMKRSSHKDGKVNLDTLGALEVDWNGITFSIGTGFDHALRDKLWSERDKLIGKIVKFKYFAQGVKTAPRFPVFIGFRDPDDM

SEQ ID NO: 51 - protein, 300 aa, Acanthocystis turfacea Chlorella virus Canal-1
MAIQKPLLAASLKKMSVGDLTFPVFATPKLDGIRALKVGGTIVSRTFKPVRNSAISEVLASILPDGSDGEILSGKTFQESTSTVMTADAGLGSGTMFFWFDYVKDDPNKGYLDRIADMKSFTDRHPEILKDKRVTIVPLFPKKIDTTEELHEFEKWCLDQGFEGVMVRNAGGKYKFGRSTEKEQILVKIKQFEDDEAVVIGVSALQTNTNDKKLNQLGEMRRTSHQDGKVELEMLGALDVDWNGIRFSIGTGFDRDTRVDLWKRREGVIGKIVKFKYFSQGIKTAPRFPVFLGFRDKDDM

SEQ ID NO: 52 - protein, 300 aa, Acanthocystis turfacea Chlorella virus Br0604L
MAIQKPLLAASLKKLSVDDLTFPVYATPKLDGIRALKIDGTLVSRTFKPIRNTTISKVLTSLLPDGSDGEILSGKTFQDSTSTVMSADAGIGSGTTFFWFDYVKDDPNKGYLDRIADIKKFIDCRPEILKDSRVIIVPLFPKKIDTAEELNVFEKWCLDQGFEGVMVRNAGGKYKFGRSTEKEQILVKIKQFEDDEAVVIGVSALQTNTNDKKVNELGEMRRTSHQDGKVDLDMLGALDVDWNGIRFGIGTGFDKDTREDLWKRRDSIIGKIVKFKYFSQGVKTAPRFPVFLGFRDKNDM

SEQ ID NO: 53 - protein, 300 aa, Acanthocystis turfacea Chlorella virus NE-JV-2
MAIQKPLLAASLKKLSVDDLTFPVYATPKLDGIRALKIDGTIVSRTFKPIRNTTISNVLMSLLPDGSDGEILSGKTFQDSTSTVMSADAGIGSGTTFFWFDYVKDDPDKGYLDRIADMKKFVDSHPEILKDRRVTIVPLIPKKIDTVEELNVFEQWCLDQGFEGVMVRNAGGKYKFGRSTEKEQILVKIKQFEDDEAVVIGVSALQTNVNDKKMNELGDMRRTSHKDGKIDLEMLGALDVEWNGIRFGIGTGFDKDTREDLWKKRDSIIGKVVKFKYFSQGIKTAPRFPVFLGFRDENDM

SEQ ID NO: 54 - protein, 300 aa, Acanthocystis turfacea Chlorella virus TN603.4.2
MAIQKPLLAASLKKMSVDNLTFPVYATPKLDGIRALKIDGTLVSRTFKPIRNTTISKVLASLLPDGSDGEILSGKTFQDSTSTVMTTDAGIGSDTTFFWFDYVKDDPDKGYLDRIADMKTFVDQHPEILKDSCVTIVPLFPKKIDTPEELHVFEKWCLDQGFEGVMVRTAGGKYKFGRSTEKEQILVKIKQFEDDEAVVIGVSALQTNTNDKKLNQLGEMRRTSHQDGKVDLDMLGALDVDWNGIRFSIGTGFDKDTREDLWKQRDSIVGKVVKFKYFSQGIKTAPRFPVFLGFRDENDM

SEQ ID NO: 55 - protein, 300 aa, Acanthocystis turfacea Chlorella virus GM0701.1
MAIQKPLLAASLKKMSVDDLTFPVYTTPKLDGIRALKIDGTLVSRTFKPVRNSAISEVLASLLPDGSDGEILSGKTFQDSTSTVMTTDAGIGSDTTFFWFDYVKDDPNKGYLDRIADMKTFIDQHPEMLKDNHVTIVPLIPKKIDTVEELNIFEKWCLDQGFEGVMVRNAGGKYKFGRSTEKEQILVKIKQFEDDEAVVIGVSALQTNTNDKKLNQLGEMRRTSHQDGKIDLEMLGALDVDWNGIRFSIGTGFDRDTRVDLWKRRDGIVGRTIKFKYFGQGIKTAPRFPVFLGFRDKDDM

SEQ ID NO: 56 - protein, 287 aa, Synechococcus phage S-CRM01
MLAGNFDPKKAKFPYCATPKIDGIRFLMVNGRALSRTFKPIRNEYIQKLLSKHLPDGIDGELTCGDTFQSSTSAIMRIAGEPDFKAWIFDYVDPDSTSILPFIERFDQISDIIYNGPIPFKHQVLGQSILYNIDDLNRYEEACLNEGYEGVMLRDPYGTYKFGRSSTNEGILLKVKRFEDAEATVIRIDEKMSNQNIAEKDNFGRTKRSSCLDGMVPMETTGALFVRNSDGLEFSIGSGLNDEMRDEIWKNKSSYIGKLVKYKYFPQGVKDLPRHPVFLGFRDPDDM

SEQ ID NO: 57 - protein, 322 aa, marine sediment metagenome
MDAHELMKLNEYAERQNQKQKKQITKPMLAASLKDITQLDYSKGYLATQKLDGIRALMIDGKLVSRTFKPIRNNHIREMLEDVLPDGADGEIVCPGAFQATSSGVMSANGEPEFIYYMFDYVKDDITKEYWRRTQDMVQWLINQGPTRTPGLSKLKLLVPTLIKNYDHLKTYETECIDKGFEGVILRTPDSPYKCGRSTAKQEWLLKLKRFADDEAVVIGFTEKMHNDNEATKDKFGHTVRSSHKENKRPAGTLGSLIVRDIKTEIEFEIGTGFDDELRQKIWDARPEWDGLCVKYKHFAISGVKEKPRFPSFIGVRDVEDM

SEQ ID NO: 58 - protein, 691 aa, Mycobacterium tuberculosis (strain ATCC 25618/H37Rv)
MSSPDADQTAPEVLRQWQALAEEVREHQFRYYVRDAPIISDAEFDELLRRLEALEEQHPELRTPDSPTQLVGGAGFATDFEPVDHLERMLSLDNAFTADELAAWAGRIHAEVGDAAHYLCELKIDGVALSLVYREGRLTRASTRGDGRTGEDVTLNARTIADVPERLTPGDDYPVPEVLEVRGEVFFRLDDFQALNASLVEEGKAPFANPRNSAAGSLRQKDPAVTARRRLRMICHGLGHVEGFRPATLHQAYLALRAWGLPVSEHTTLATDLAGVRERIDYWGEHRHEVDHEIDGVVVKVDEVALQRRLGSTSRAPRWAIAYKYPPEEAQTKLLDIRVNVGRTGRITPFAFMTPVKVAGSTVGQATLHNASEIKRKGVLIGDTVVIRKAGDVIPEVLGPVVELRDGSEREFIMPTTCPECGSPLAPEKEGDADIRCPNARGCPGQLRERVFHVASRNGLDIEVLGYEAGVALLQAKVIADEGELFALTERDLLRTDLFRTKAGELSANGKRLLVNLDKAKAAPLWRVLVALSIRHVGPTAARALATEFGSLDAIAAASTDQLAAVEGVGPTIAAAVTEWFAVDWHREIVDKWRAAGVRMVDERDESVPRTLAGLTIVVTGSLTGFSRDDAKEAIVARGGKAAGSVSKKTNYVVAGDSPGSKYDKAVELGVPILDEDGFRRLLADGPASRT

SEQ ID NO: 59 - protein, 676 aa, Enterococcus faecalis (strain ATCC 700802/V583)
MEQQPLTLTAATTRAQELRKQLNQYSHEYYVKDQPSVEDYVYDRLYKELVDIETEFPDLITPDSPTQRVGGKVLSGFEKAPHDIPMYSLNDGFSKEDIFAFDERVRKAIGKPVAYCCELKIDGLAISLRYENGVFVRGATRGDGTVGENITENLRTVRSVPMRLTEPISVEVRGECYMPKQSFVALNEEREENGQDIFANPRNAAAGSLRQLDTKIVAKRNLNTFLYTVADFGPMKAKTQFEALEELSAIGFRTNPERQLCQSIDEVWAYIEEYHEKRSTLPYEIDGIVIKVNEFALQDELGFTVKAPRWAIAYKFPPEEAETVVEDIEWTIGRTGVVTPTAVMAPVRVAGTTVSRASLHNADFIQMKDIRLNDHVIIYKAGDIIPEVAQVLVEKRAADSQPYEMPTHCPICHSELVHLDEEVALRCINPKCPAQIKEGLNHFVSRNAMNIDGLGPRVLAQMYDKGLVKDVADLYFLTEEQLMTLDKIKEKSANNIYTAIQGSKENSVERLIFGLGIRHVGAKAAKILAEHFGDLPTLSRATAEEIVALDSIGETIADSVVTYFENEEVHELMAELEKAQVNLTYKGLRTEQLAEVESPFKDKTVVLTGKLAQYTREEAKEKIENLGGKVTGSVSKKTDIVVAGEDAGSKLTKAESLGVTVWNEQEMVDALDASHF

SEQ ID NO: 60 - protein, 670 aa, Haemophilus influenzae (strain ATCC 51907/DSM 11121/ KW20/Rd)
MTNIQTQLDNLRKTLRQYEYEYHVLDNPSVPDSEYDRLFHQLKALELEHPEFLTSDSPTQRVGAKPLSGFSQIRHEIPMLSLDNAFSDAEFNAFVKRIEDRLILLPKPLTFCCEPKLDGLAVSILYVNGELTQAATRGDGTTGEDITANIRTIRNVPLQLLTDNPPARLEVRGEVFMPHAGFERLNKYALEHNEKTFANPRNAAAGSLRQLDPNITSKRPLVLNAYGIGIAEGVDLPTTHYARLQWLKSIGIPVNPEIRLCNGADEVLGFYRDIQNKRSSLGYDIDGTVLKINDIALQNELGFISKAPRWAIAYKFPAQEELTLLNDVEFQVGRTGAITPVAKLEPVFVAGVTVSNATLHNGDEIERLNIAIGDTVVIRRAGDVIPQIIGVLHERRPDNAKPIIFPTNCPVCDSQIIRIEGEAVARCTGGLFCAAQRKEALKHFVSRKAMDIDGVGGKLIEQLVDRELIHTPADLFKLDLTTLTRLERMGAKSAENALNSLENAKSTTLARFIFALGIREVGEATALNLANHFKTLDALKDANLEELQQVPDVGEVVANRIFIFWREAHNVAVVEDLIAQGVHWETVEVKEASENLFKDKTVVLTGTLTQMGRNEAKALLQQLGAKVSGSVSSKTDFVIAGDAAGSKLAKAQELNITVLTEEEFLAQITR

SEQ ID NO: 61 - protein, 667 aa, Staphylococcus aureus
MADLSSRVNELHDLLNQYSYEYYVEDNPSVPDSEYDKLLHELIKIEEEHPEYKTVDSPTVRVGGEAQASFNKVNHDTPMLSLGNAFNEDDLRKFDQRIREQIGNVEYMCELKIDGLAVSLKYVDGYFVQGLTRGDGTTGEDITENLKTIHAIPLKMKEPLNVEVRGEAYMPRRSFLRLNEEKEKNDEQLFANPRNAAAGSLRQLDSKLTAKRKLSVFIYSVNDFTDFNARSQSEALDELDKLGFTTNKNRARVNNIDGVLEYIEKWTSQRESLPYDIDGIVIKVNDLDQQDEMGFTQKSPRWAIAYKFPAEEVVTKLLDIELSIGRTGVVTPTAILEPVKVAGTTVSRASLHNEDLIHDRDIRIGDSVVVKKAGDIIPEVVRSIPERRPEDAVTYHMPTHCPSCGHELVRIEGEVALRCINPKCQAQLVEGLIHFVSRQAMNIDGLGTKIIQQLYQSELIKDVADIFYLTEEDLLPLDRMGQKKVDNLLAAIQQAKDNSLENLLFGLGIRHLGVKASQVLAEKYETIDRLLTVTEAELVEIHDIGDKVAQSVVTYLENEDIRALIQKLKDKHVNMIYKGIKTSDIEGHPEFSGKTIVLTGKLHQMTRNEASKWLASQGAKVTSSVTKNTDVVIAGEDAGSKLTKAQSLGIEIWTEQQFVDKQNELNS

SEQ ID NO: 62 - protein, 652 aa, Streptococcus pneumoniae (strain P1031)
MNKRMNELVALLNRYATEYYTSDNPSVSDSEYDRLYRELVELETAYPEQVLADSPTHRVGGKVLDGFEKYSHQYPLYSLQDAFSREELDAFDARVRKEVAHPTYICELKIDGLSISLTYEKGILVAGVTRGDGSIGENITENLKRVKDIPLTLPEELDITVRGECYMPRASFDQVNQARQENGEPEFANPRNAAAGTLRQLDTAVVAKRNLATFLYQEASPSTRDSQEKGLKYLEQLGFVVNPKRILAENIDEIWNFIQEVGQERENLPYDIDGVVIKVNDLASQEELGFTVKAPKWAVAYKFPAEEKEAQLLSVDWTVGRTGVVTPTANLTPVQLAGTTVSRATLHNVDYIAEKDIRKDDTVIVYKAGDIIPAVLRVVESKRVSEEKLDIPTNCPSCNSDLLHFEDEVALRCINPRCPAQIMEGLIHFASRDAMNITGLGPSIVEKLFAANLVKDVADIYRLQEEDFLLLEGVKEKSAAKLYQAIQASKENSAEKLLFGLGIRHVGSKASQLLLQYFHSIENLYQADSEEVASIESLGGVIAKSLQTYFATEGSEILLRELKETGVNLDYKGQTVVADAALSGLTVVLTGKLERLKRSEAKSKLESLGAKVTGSVSKKTDLVVVGADAGSKLQKAQELGIQVRDEAWLESL

SEQ ID NO: 63 - protein, 374 aa, Wild-type Enterobacteria phage T4 RNA ligase 1 protein sequence - 'Rnl1'
MQELFNNLMELCKDSQRKFFYSDDVSASGRTYRIFSYNYASYSDWLLPDALECRGIMFEMDGEKPVRIASRPMEKFFNLNENPFTMNIDLNDVDYILTKEDGSLVSTYLDGDEILFKSKGSIKSEQALMANGILMNINHHRLRDRLKELAEDGFTANFEFVAPTNRIVLAYQEMKIILLNVRENETGEYISYDDIYKDATLRPYLVERYEIDSPKWIEEAKNAENIEGYVAVMKDGSHFKIKSDWYVSLHSTKSSLDNPEKLFKTIIDGASDDLKAMYADDEYSYRKIEAFETTYLKYLDRALFLVLDCHNKHCGKDRKTYAMEAQGVAKGAGMDHLFGIIMSLYQGYDSQEKVMCEIEQNFLKNYKKFIPEGY

SEQ ID NO: 64 - protein, 334 aa, Wild-type Enterobacteria phage T4 RNA ligase 2 protein sequence - 'Rnl2'
MFKKYSSLENHYNSKFIEKLYSLGLTGGEWVAREKIHGTNFSLIIERDKVTCAKRTGPILPAEDFFGYEIILKNYADSIKAVQDIMETSAVVSYQVFGEFAGPGIQKNVDYCDKDFYVFDIIVTTESGDVTYVDDYMMESFCNTFKFKMAPLLGRGKFEELIKLPNDLDSVVQDYNFTVDHAGLVDANKCVWNAEAKGEVFTAEGYVLKPCYPSWLRNGNRVAIKCKNSKFSEKKKSDKPIKAKVELSEADNKLVGILACYVTLNRVNNVISKIGEIGPKDFGKVMGLTVQDILEETSREGITLTQADNPSLIKKELVKMVQDVLRPAWIELVS

SEQ ID NO: 65 - protein, 389 aa, Wild-type Aeromonas virus Aeh1 ligase protein sequence - 'RNA3'
MQSIKELYQNLINLCVDDNTKFYFAETVTSLGTKVRIFDYHVAGYNDWIRPDAMASRGIMFEMNGEIPVRIMSRPMDKFFNYSEVIGWEKLETAGNMKMPDLNKIAYVIDKRDGSLISTYLDISGEIKNLLLKSKASIRSNQANDASVWLYQEDHKDLLEFCTAYAENGFTVNMEWTAPHNQIVLCYNEHQLRILNIRHNETGEYVDFGELQKDPTFVKYAADFFEVPGDGKAWIDEVYQMTGIEGFVVVMEDYQMFKLKTDWYVALHHTKDSINNSERLIYACAENCTDDLRQMFRDDENSLQKIEIFDNHFRDVVMDAMKKLTEAYEKYRGMERRDYAINMNNDFKNERHWFNIAMQMFAQRPDFSMTDEIVAVIKKYPKTFIPKGY

SEQ ID NO: 66 - protein, 383 aa, Wild-type Klebsiella phage JD18 ligase protein sequence - 'RNA6'
MLELYKNLMNLCESSEVAKFFYKDFTGPMDGKFRVFSYHYASYSEWLKPDALECRGIMFEMDGDTPIRIASRPMEKFFNLNENPMTMGIDISDVEYIMDKADGSLVSSYVDDGYLYLKSKTSLYSDQARQASALLNSEEYSSLHQVILELALDGYTVNMEFVSPNNRVVLAYQEPQLFVLNVRNNTTGEYIKYDDLYANAKIRPYLINAYGISDPTTWVEGVRALEGVEGYIAVLNTGQRFKVKTEWYSALHHTKDSITSNERLFASVVSANSDDLRSLFAGDEYAIKKISAFEQAYLDYLGKSLELCQSFYDEYRGRARKDYAIAAQKATVNQRHLFGVIMNMYEGTVDVDKLLKDLERVFLKYWAGYVPKEYEKEIEISEE

SEQ ID NO: 67 - protein, 384 aa, Wild-type Stenotrophomonas phage IME13 ligase protein sequence - 'RNA8'
MSRTIELFNNLMSVVEKSEKGNFYFKDVITSMGTKARIFSYFIASYTDWLQDDALECRGIMFELNDKNEPVRIMARPMQKFFNLKENPMTIGLDLTKMIGLMEKADGSLISSYHDQGYVYLKSKAAIFSDQANKAMALLNSPAYEKLRDAIVRAGSDFTFNMEYVGPSNRVVLPYEEEELIVLNVRHNETGQYVEFSTLLDDPLIRHRMIGVYPCPDWSKVTPEEWEAATRAETDIEGVIGIMPDGQLFKLKTDWYSSLHRTKDSINNNKALFQSIKERASDDLRGMFSDDNAALAKIEAFESAYIDTVAKYHKICAEVFLRFARFLIVEVFAIEAQARMKDCRYLFSIVMQQYGRDWDGELAVEKIEEHIIKEYATYVPMAYR

SEQ ID NO: 68 - protein, 394 aa, Wild-type Escherichia phage JSE ligase protein sequence - 'RNA9'
MEHKLCQQKKTTKKVLALFKNLMALCDGSDTFYYKDEITAMQTRMRIFSYLYLSKPEMWNKPDALECRGIMFEIDDKDRPVRIASRPMEKFFNLGENDRARFKPEDVEMVMDKMDGSLVSTYIDNGYVQLKSKAALYSSQAERANGLLYSEKYADLRAKIADIGSDYTFNFEYTAPSNRIVVEYSEPSLTLLNVRHNVTGEYVPHQMLFADAILRPHLVNALQVDSARFSNILDEVRTAEGIEGIVARTKDGQMFKVKSEWYIGVHNIKNTSMFPNNLIYYVVESETDDLRAAYEGEPEALERIELFEEAFRSILRNAFTTATEFYNAHAGEDRKTYASNATIESRKHGDAQSYIFMCLMIAFDGLDYDRILASMKTYYLRNYKKLIPADKIDW

SEQ ID NO: 69 - protein, 385 aa, Wild-type Acinetobacter phage Acj61 ligase protein sequence - 'RNA16'
MKELFDNLMALQDPNDISKFFYKDVVTQPGTKCRIFSYNYAAYSDWLLPGALESRGIMFELDADNQPVRVMARPMEKFFNLEENPFTMDLDLSQLEYAMTKADGSLISTYVDQGYLYTKSKGSISSSQAIESKQLLLDINYKPLAERALELAKDGFTCNFEYVAPNNRIVLNYAKKDLILLNVRHNETGEYVPMAELQKDPVLRNYLIDVYPPREDIDTNEMIKEIREMVDIEGFVFQHASGLKFKLKTEWYSNLHRVKDTLNNSEALFMVVVAGGSDDMKSLFTDDLSRTKIESFETAFLDYLKKTSNFVFDLQRQLIGSDRKTYAIECQTILRNTDQLELFGVMMELYKGADQEQTIKNINVVFMKNYKKYVPAGFETLKNEY

SEQ ID NO: 70 - protein, 381 aa, Wild-type Vibrio phage VH7D ligase protein sequence - 'RNA20'
MNVQELYKNLMSLADDAEGKFFFADHLSPLGEKFRVFSYHIASYSDWLLPGALEARGIMFQLDDNDEMIRIVSRPMEKFFNLNENPFTMELDLTTTVQLMDKADGSLISTYLSGENFALKSKTSIFSEQAVAANRYIKKPENRDLWEFCDDCTQAGLTVNMEWCAPNNRIVLEYPEAKLVILNIRDNETGDYVSFDDIPQSALMRVKQWLVDEYDPATAHEPDFVEKLRDTKGIEGMILRLANGQSVKIKTQWYVDLHSQKDSVNVPKKLVTTILNGNHDDLYALFADDKPTIERIREFDSHVTKTLTNSFNAVRQFYARNRHLARKDYAIAGQKVLKPWEFGVAMIAYQKQTVEGVYESLVTAYLKRPELAIPEKYLNGV

SEQ ID NO: 71 - protein, 382 aa, Wild-type Escherichia phage JS98 ligase protein sequence - 'RNA22'
MIELYDNLMTLVKNSTKSKFFFKDFQSALGVNYRIFSYNYASYSDWLEDGALECRGIMFEMDENGPVRIAARPMQKFFNLDENPLTIGLDLSQENIDLVMAKEDGSLISTFMDRQYLSVKSKGSIHSSMVHDSLRFLRLPENEAFAARLEEITKAGYTCNLEYVSPTNRIVLAYQETNLILLNVRNNETGEYIPYAELFKDGALRKHLVKSYELSEGDFVDNIRKQEGIEGFIFVLKDGTFFKLKTAWYSALHHTKDSINNNERLFEVVVAGGTDDLRGLFSTDSFAIEKINAFERIHLDYLEQSLALLEAAYSQLKGRDRKDYAVTGQLILKDFPGLFSILMQAYVDGINYDTVMDQINSVFLKNHKAQIPEKYLKEIVVE

SEQ ID NO: 72 - protein, 386 aa, Wild-type Escherichia phage vB_EcoM_112 ligase protein sequence - 'RNA23'
MVLYSKHKRGYTMQELFNNLMELCKDSQRKFFYSDDVSASGRTYRIFSYNYASYSDWLLPDALECRGIMFEMDGEKPVRIASRPMEKFFNLNENPFTMNIDLNDVDYILTKEDGSLVSTYLDGDEILFKSKGSIKSEQALMANGILMNINHHQLRDRLKELAEDGFTANFEFVAPTNRIVLAYQEMKIILLNVRENETGEYISYDDIYKDAILRPYLVERYEIDSPKWVEEAKNAENIEGYVAVMKDGSHFKIKSDWYVSLHSTKSSLDNPEKLFKTIIDGASDDLKAMYADDEYSYRKIEAFETTYLKYLDRALFLVLDCHNKHCGKDRKTYAMEAQGVAKGAGMDHLFGIIMSLYQGYDSQEKVMCEIEQNFLKNYKKFIPEGY

SEQ ID NO: 73 - protein, 392 aa, Wild-type Aeromonas phage CC2 ligase protein sequence - 'RNA28'
MKELYNNLLKLTEEHGDCFFFRDHWSSIGNHFRVFSYHIAGLTQWMLPDALECRGIMFELINGEPYRIASRPMEKFFNLAERQAWNLTNSGVVGLDKLELDYSNIDRYEDKADGSLMSSYHFIDPEDDNRINYMLKSKTSINSDQANDANRWLVNHTDLLDFIIDCEEAGYTVNLEWCSPKNQIVIMYPEESLKILNVRHRDTGEYYSNNSLIRSPVFRKYAVDQFMFEEGTDVNTAISNMYNETGIEGYILVMRDGSRVKIKTTSYVARHKLKDSITNNKDLVIAVAQGVSDDLRQLFLDDSLSLTKIQEFEDHVVSVAGSTYTKIREAHKACAGMERREYAISMQNTFKQDRMFFNIVMKMFQAPDLEVMPEIMSVIIKYPDEFVPTKWK

SEQ ID NO: 74 - protein, 374 aa, Wild-type Enterobacteria phage RB69 ligase protein sequence - 'RNA29'
MEKLYYNLLSLCKSSSDRKFFYSDDVSPIGKKYRIFSYNFASYSDWLLPDALECRGIMFEMDGETPLRIASRPMEKFFNLNENPFTLSIDLNDVKYLMTKEDGSLVSTYLDGNMVRFKSKGSIKSDQAASATSILLDINHKDLADRLLELCNDGFTANFEYVAPSNKIVLTYPEKRLILLNIRDNNTGKYIEYDDIYLDPVFRKYLVDRFEAPEGDWVPGVKSSTNIEGYVAVMKDGSHFKLKTDWYVALHTTRDSISSPEKLFLAIMNGASDDLKAMYADDEFSFKKVELFEKAYLDFLDRSFYICLDAYDKHKGKDRKTYAIEAQAICKGAQSPWLFGIIMNLYQGGSKEQMMTALESVFIKNHKNFIPEGY

SEQ ID NO: 75 - protein, 388 aa, Wild-type Acinetobacter phage Ac42 ligase protein sequence - 'RNA31
MNELYNNLMTLIEPGKMSRFFLRDAVTPFGTRVRMFGYNYASYTDWLLPDALEARGIMFEMDENDQPIRVMARPMEKFFNLGENPFTIDLDLSTIEYFMDKSDGSLISSYVDNDTLFMKSKMSIGSVQAVAARQVIQDYVHRDLHDRVLELAKDGFTCNFEYVAPDNRVVILYPERALVLLNVRNNETGEYVHIEELKRDPVLRRYLVNNYVIDPENFDQDTFVNDIYQMVDIEGYVFRLMTGQHVKIKTEWYKMLHYAKDTINNNEALFAITVAAQLDDVRSLYSDDYALGKINKFEEVFLGFLDTRLPILLNLHKELNGSSRKDYAIKSQTYFKQANELYLFGIFMQMFEGVPPREQLVEKLSEAFMKNYKLFVPPEYDKVVEYDN

SEQ ID NO: 76 - protein, 382 aa, Wild-type Pectobacterium phage CBB ligase protein sequence - 'RNA33'
MRTKQIFDDLMNLTAKNDAFMWKDFVSPAGGLFRIFSYRLASYSDFLEPNALECRGSMFKVDDEGNFVGIASRTPMKFFNAYENPFTMYDKDTLSSEIAVVMDKLDGSIISTFMDVDFVVRTKSHASLHSDHAYNSTAMLIADKELYNEVHYAESMGYTVNMEYTSPEYRIVLPYQEDNLTVLNLRHRETGELLIGERLKEFSKILYERSVFAKHGEIDATFPMKETLKESIDAVRGMADIEGYVLILKDGRMCKIKTDWYCALHFTKDSINVDSRLYDAIITGASDDLKQMFSTDLYAMKKIEKMEQLIFSCYNKLVHDVESFYEENKHLERKEYALKVQSTLPNELGMPGLAFSLYASKPVDYKGQMLKYMKDVLVNFEV

SEQ ID NO: 77 - protein, 385 aa, Wild-type Aeromonas phage phiAS5 ligase protein sequence - 'RNA35
MQSIKELYQNLVNLCVDDNTKFFFSETVTSLGTKVRIFDYHVAGYNDWIRPDAMACRGIMFEMNGEIPVRIMSRPMDKFFNYSEVIGWEKLETHGNMKMPDLSKIKFVIDKRDGSLISTFMDVDNLLLKSKGSIRSNQANDASVWLYQDDQADLLEFCRAYAKEGFTVNMEWTAPHNQIVLCYTDHQLRILNIRHNETGEYVDFAELQKDSVFRKYAADFYEVPQDGAEWIKNVYGMTGIEGYVVVMEDYQMFKLKTDWYVALHHTKDSINDSKRLISACAENATDDLRQMFRDDPNSLAKIEVFDAKFRDVVSSAMQALTNAYSKYKALERREYAISMTNEFKNERHWFNIAMQMFSTRPDFSLADEIVAVIKKYPEKFVPQGY

SEQ ID NO: 78 - protein, 376 aa, Wild-type Salmonella phage vB_SenMS16 ligase protein sequence - 'RNA36
MKELFDNLMNLCNDTDESRFFYRDDISPSGLKYRIFSYNYASYSDWLLPDALECRGIMFEMIDGVPVRIASRPMEKFFNLNETPFTMNLDLSNAVHMMKKEDGSLVSSYLDGNILRFKSKSSLKSEQAYLSSAMLTSITHEALLWRLLELARDGFTANFEYVSPENRIVLAYQKKDLILLNIRENDTGAYVPYNEIAKDPVLRQYLVESYEIPEGDFVSDIKAMEGIEGYVFVMDNGLRFKLKTDWYTALHHTKDSITKNDRLFEVIVNNASDDLKGLFSNDAYSLKKINKFEEVYLDYLRRSLSFISTSYQKLRGLDRKTYAGEAKRLADAERLPFLFTILMLMFNDSMDYDTTIKKVNELFMKNYKTFIPKEYE

SEQ ID NO: 79 - protein, 381 aa, Wild-type Vibrio phage KVP40 ligase protein sequence - 'RNA39'
MTTQELYNHLMTLTEDAEGKFFFADHISPLGEKLRVFSYHIASYSDWLLPGALEARGIMFQLDEQDKMVRIVSRPMEKFFNLNENPFTMDLDLTTTVQLMDKADGSLISTYLTGENFALKSKTSIFSEQAVAANRYIKLPENRDLWEFCDDLTQAGCTVNMEWCAPNNRIVLEYPEAKLVILNIRDNETGDYVSFDDIPLPALMRVKKWLVDEYDPETAHVDDFVEKLRATKGIEGMILRLANGQSVKIKTQWYVDLHSQKDSVNVPKKLVTTILNNNHDDLYALFADDKPTIDRIREFDSHVSKTVSASFHAVSQFYVKNRHMSRKDYAIAGQKALKPWEFGVAMIAYQKKTVEGVYEALVGAYLKRPELLIPEKYLNEA

SEQ ID NO: 80 - protein, 361 aa, Wild-type Campylobacter virus CP220 ligase protein sequence - 'RNA49'
MNYLELKNMAENLKDSNYRSTKLNNFKFYTYIFSDYKNFKENNTFFIRGLMIDSKSILNKDTLAPGISIPMPKFFNINENEDWLLPDSTNLEDFTIVTKYDGSLMIPYEYDGIKFRTKMSIDNDQTKLANKYIKNNPDILDLIKNNPDTQYFFELISPLNRIVVDYNKTELKLIAELDLRTLEFKIHETNEFNFKDLNIKTLKDLKDYINTISNYEGVILQHKVTKKVYKLKTQEYLDLHNTMTNLDLKVIYKMILEETIDDVLPKLSPEAVAYIDSVSNSVKVKLNEILDSIDSNYIKTKDLETPALYIKDLNIDPIAKDCLFKLCKNKLNLDDVLNQVKKSMLKYNKLRDIKVFLKWIH

SEQ ID NO: 81 - protein, 380 aa, Wild-type Pseudomonas phage phiPMW ligase protein sequence - 'RNA59'
MKVIEFLKNAPSITDGLASLHLELGIKAKIYEDEGLIVLNYSQIDSPKTHPIVQECRGLIIDNDLTVVARPFDRFFNYGEALNVMPEIDWENASIFEKVDGSLIKIYFHKGRWEVATRGTAFAESECMGHGITFKELVFNALKVHDDDGFQYLMNNAYLFRDTTYLFELTCVENRVVRHYHGYNLHFLAARDNVSGNYSEECRDWLRSPDCILYGIVKHPKRYALGSADEALQAAKELKNLDEGFIVYQNAVPIAKIKSPAYVAVHHIRGEGLNPKRIMELVLSGEHDEYLSYFPEDRPIIQPYVDSLLDMLNIIAVTYPRLNQATTPKAFAAAIKHAGIDKQKASVYFMARRDNKDPVQVFHGMKTTFKMDMLRKWMMV

SEQ ID NO: 82 - protein, 317 aa, Wild-type Pseudomonas phage vB_PaeM_C2-10_Ab1 ligase protein sequence - 'RNA61'
MPNCRIEIRRSRMEGNLNIAMYKDLIANKLVTVKHFNGMSIIKYARKVFYENLWNEHPLLLEARGHVFDQHSGDCIVRPFEKVFNLGENGAGSFLHPKFRVRLIEKVNGFMFSVTKHNGSLIFSTTGSLTSDYVALGQKYVSNNPDDYIAGFTYNFEICSPDDPHIVEEEEGAYLIGIRDIFTGGQLSEYILDSHALGVTDHSSVKILRPEHIECSWEHAKGLLSSCEKEGYMVQTGLGTVKCKSTHYLGKKFIMRMGSKKVNSMYQDPAGFKQTLDEEFYPLVDFLVNEVEEVRFTEMTDAQRRLLIETYFDMARI

SEQ ID NO: 83 - protein, 368 aa, Wild-type Butyrivibrio proteoclasticus ligase protein sequence - 'RNA82'
MKSRILEFIKNNPDTWEEKLNEKFIRTNHNGDLVCFKYATEADFSDPLVCEARGIIIDVAQLVVVCWPFDKFFNVQEKYAADIDWNSARVLEKIDGSMIKLFWYKGAWRFATSSTCDAKDAAIPGYNELTYADIIARAENVNEIPFEELNKDYTYIFELVSPLSQIVVRYEMTELFFLTARNNLTGEELDTELLQFRRPRSFALKSMNECLDAALALNKGDEIEDEGFVVVDEKHNRVKIKSPAYVAMHRLSTNKVFTVKRMAEFFCNGEDLSKLAKDFPANAHIIKYYDWQFAEMKHKAEDMMLYSRRLYEEYDHDRKAVAMTIKDSPYAWAGFRAIGNDKDITDIMAVLAPANVEKLIVEYPEISN

SEQ ID NO: 84 - RNA, 10 nt, Artificial Sequence
  Example 15 and 16 primer oligonucleotide sequence
acuccucggu

SEQ ID NO: 85 - RNA, 11 nt, Artificial Sequence
  Example 15 and 16 product oligonucleotide sequence
acuccucggua

SEQ ID NO: 86 - DNA, 10 bp, Artificial Sequence
  Example 17 primer oligonucleotide sequence
actcatcgat

SEQ ID NO: 87 - DNA, 11 bp, Artificial Sequence
  Example 17 product oligonucleotide sequence
actcatcgata

SEQ ID NO: 88 - protein, 384 aa, Artificial Sequence
  Mutant ligase (Stenotrophomonas phage IME13 backbone) protein sequence
MSRTIELFNNLMSVVEKSEKGNFYFKDVITSMGTKARIFSHKIASYTDWLQDDALECRGIMFELNDKNEPVRIMARPMQKFFNLKENPMTIGLDLTKMIGLMEKADGSLISSYHDQGYVYLKSKTSIFSDQANKAMALLNSPAYEKLRDAIVRAGSDFTFNMEYVGPSNRVVLPYEEEELIVLNVRHNETGQYVEFSTLLDDPLIRHRMIGVYPCPDWSKVTPEEWEAATRAETDIEGVIGIMPDGQLFKLKTDWYSSLGRTKFSINNNKALHQSIKERASVALRGMFSDDNAALAKIEAFESAYIDTVAKYHKICAEVFLRFARFLIVEVFAIEAQARMKDCRYLFSIVMQQYGRDWDGELAVEKIEEHIIKEYATYVPMAYR

SEQ ID NO: 89 - protein, 384 aa, Artificial Sequence
  Mutant ligase (Stenotrophomonas phage IME13 backbone) protein sequence
MSRTIELFNNLMSVVEKSEKGNFYFKDVITSMGTKARIFSHQIASYTDWLQDDALECRGIMFELNDKNEPVRIMARPMQKFFNLKENPMTIGLDLTKMIGLMEKADGSLISSYHDQGYVYLKSKTSIFSDQANKAMALLNSPAYEKLRDAIVRAGSDFTFNMEYVGPSNRVVLPYEEEELIVLNVRHNETGQYVEFSTLLDDPLIRHRMIGVYPCPDWSKVTPEEWEAATRAETDIEGVIGIMPDGQLFKLKTDWYSSLGRTKFSINNNKALHQSIKERASGALRGMFSDDNAALAKIEAFESAYIDTVAKYHKICAEVFLRFARFLIVEVFAIEAQARMKDCRYLFSIVMQQYGRDWDGELAVEKIEEHIIKEYATYVPMAYR

SEQ ID NO: 90 - protein, 384 aa, Artificial Sequence
  Mutant ligase (Stenotrophomonas phage IME13 backbone) protein sequence
MSRTIELFNNLMSVVEKSEKGNFYFKDVITSMGTKARIFSYFIASYTDWLQDDALECRGIMFELNDKNEPVRIMARPMQKFFNLKENPMTIGLDLTKMIGLMEKADGSLISSYHDQGYVYLKSKTSIFSDQANKAMALLNSPAYEKLRDAIVRAGSDFTFNMEYVGPSNRVVLPYEEEELIVLNVRHNETGQYVEFSTLLDDPLIRHRMIGVYPCPDWSKVTPEEWEAATRAETDIEGVIGIMPDGQLFKLKTDWYSSLGRTKYSINNNKALNQSIKERASVALRGMFSDDNAALAKIEAFESAYIDTVAKYHKICAEVFLRFARFLIVEVFAIEAQARMKDCRYLFSIVMQQYGRDWDGELAVEKIEEHIIKEYATYVPMAYR

SEQ ID NO: 91 - protein, 384 aa, Artificial Sequence
  Mutant ligase (Stenotrophomonas phage IME13 backbone) protein sequence
MSRTIELFNNLMSVVEKSEKGNFYFKDVITSMGTKARIFSHNIASYTDWLQDDALECRGIMFELNDKNEPVRIMARPMQKFFNLKENPMTIGLDLTKMIGLMEKADGSLISSYHDQGYVYLKSKTTIFSDQANKAMALLNSPAYEKLRDAIVRAGSDFTFNMEYVGPSNRVVLPYEEEELIVLNVRHNETGQYVEFSTLLDDPLIRHRMIGVYPCPDWSKVTPEEWEAATRAETDIEGVIGIMPDGQLFKLKTDWYSSLGRTKYSINNNKALHQSIKERASVDLRGMFSDDNAALAKIEAFESAYIDTVAKYHKICAEVFLRFARFLIVEVFAIEAQARMKDCRYLFSIVMQQYGRDWDGELAVEKIEEHIIKEYATYVPMAYR

SEQ ID NO: 92 - protein, 384 aa, Artificial Sequence
  Mutant ligase (Stenotrophomonas phage IME13 backbone) protein sequence
MSRTIELFNNLMSVVEKSEKGNFYFKDVITSMGTKARIFSHKIASYTDWLQDDALECRGIMFELNDKNEPVRIMARPMQKFFNLKENPMTIGLDLTKMIGLMEKADGSLISSYHDQGYVYLKSKAAIFSDQANKAMALLNSPAYEKLRDAIVRAGSDFTFNMEYVGPSNRVVLPYEEEELIVLNVRHNETGQYVEFSTLLDDPLIRHRMIGVYPCPDWSKVTPEEWEAATRAETDIEGVIGIMPDGQLFKLKTDWYSSLHRTKDSINNNKALFQSIKERASDDLRGMFSDDNAALAKIEAFESAYIDTVAKYHKICAEVFLRFARFLIVEVFAIEAQARMKDCRYLFSIVMQQYGRDWDGELAVEKIEEHIIKEYATYVPMAYR

SEQ ID NO: 93 - DNA, 11 bp, Artificial Sequence
  Example 26 product oligonucleotide sequence
actcatcgatc

SEQ ID NO: 94 - DNA, 11 bp, Artificial Sequence
  Example 26 product oligonucleotide sequence
actcatcgatt

SEQ ID NO: 95 - protein, 477 aa, Wild type phosphatase (Pandalus borealis) protein sequence - 'SAP'
MEEDKAYWNKDAQDALDKQLGIKLREKQAKNVIFFLGDGMSLSTVTAARIYKGGLTGKFEREKISWEEFDFAALSKTYNTDKQVTDSAASATAYLTGVKTNQGVIGLDANTVRTNCSYQLDESLFTYSIAHWFQEAGRSTGVVTSTRVTHATPAGTYAHVADRDWENDSDVVHDREDPEICDDIAEQLVFREPGKNFKVIMGGGRRGFFPEEALDIEDGIPGEREDGKHLITDWLDDKASQGATASYVWNRDDLLAVDIRNTDYLMGLFSYTHLDTVLTRDAEMDPTLPEMTKVAIEMLTKDENGFFLLVEGGRIDHMHHANQIRQSLAETLDMEEAVSMALSMTDPEETIILVTADHGHTLTITGYADRNTDILDFAGISDLDDRRYTILDYGSGPGYHITEDGKRYEPTEEDLKDINFRYASAAPKHSATHDGTDVGIWVNGPFAHLFTGVYEENYIPHALAYAACVGTGRTFCD

SEQ ID NO: 96 - DNA, 11 bp, Artificial Sequence
  Example 27 product oligonucleotide sequence
actcatcgata

SEQ ID NO: 97 - DNA, 12 bp, Artificial Sequence
  Example 27 product oligonucleotide sequence
actcatcgataa

SEQ ID NO: 98 - DNA, 12 bp, Artificial Sequence
  Example 27 product oligonucleotide sequence
actcatcgataa

SEQ ID NO: 99 - DNA, 12 bp, Artificial Sequence
  Example 28 product oligonucleotide sequence
  misc_feature (4)..(4): n = 2' deoxyInosine
actnagaccacg

SEQ ID NO: 100 - protein, 221 aa, Wild type Archaeoglobus fulgidus endonuclease V endonuclease
MLQMNLEELRRIQEEMSRSVVLEDLIPLEELEYVVGVDQAFISDEVVSCAVKLTFPELEVVDKAVRVEKVTFPYIPTFLMFREGEPAVNAVKGLVDDRAAIMVDGSGIAHPRRCGLATYIALKLRKPTVGITKKRLFGEMVEVEDGLWRLLDGSETIGYALKSCRRCKPIFISPGSYISPDSALELTRKCLKGYKLPEPIRIADKLTKEVKRELTPTSKLK

SEQ ID NO: 101 - DNA, 7 bp, Artificial Sequence
  Example 28 product oligonucleotide sequence
gaccacg